European Patent Specification EP 3 609 920 B1, published July 12, 2023. Title: ANTI-PD-L1-ANTI-TIM-3 BISPECIFIC ANTIBODIES. Applicant: Eli Lilly and Company Zymeworks, Inc. The sequence listing filed with the application follows.

SEQUENCE LISTING (32 sequences)

SEQ ID NO: 1 - protein, 290 aa, Homo sapiens
MRIFAVFIFMTYWHLLNAFTVTVPKDLYVVEYGSNMTIECKFPVEKQLDLAALIVYWEMEDKNIIQFVHGEEDLKVQHSSYRQRARLLKDQLSLGNAALQITDVKLQDAGVYRCMISYGGADYKRITVKVNAPYNKINQRILVVDPVTSEHELTCQAEGYPKAEVIWTSSDHQVLSGKTTTTNSKREEKLFNVTSTLRINTTTNEIFYCTFRRLDPEENHTAELVIPELPLAHPPNERTHLVILGAILLCLGVALTFIFRLRKGRMMDVKKCGIQDTNSKKQSDTHLEET

SEQ ID NO: 2 - protein, 130 aa, Homo sapiens
MFSHLPFDCVLLLLLLLLTRSSEVEYRAEVGQNAYLPCFYTPAAPGNLVPVCWGKGACPVFECGNVVLRTDERDVNYWTSRYWLNGDFRKGDVSLTIENVTLADSGIYCCRIQIPGIMNDEKFNLKLVIK

SEQ ID NO: 3 - protein, 123 aa, Artificial Sequence
  synthetic construct
QVQLVQSGAEVKKPGSSVKVSCKASGGTFSSYAISWVRQAPGQGLEWMGGIIPIFGTANYAQKFQGRVTITADKSTSTAYMELSSLRSEDTAVYYCARSPDYSPYYYYGMDVWGQGTTVTVSS

SEQ ID NO: 4 - protein, 111 aa, Artificial Sequence
  synthetic construct
QSVLTQPPSASGTPGQRVTISCSGSSSNIGSNTVNWYQQLPGTAPKLLIYGNSNRPSGVPDRFSGSKSGTSASLAISGLQSEDEADYYCQSYDSSLSGSVFGGGIKLTVLG

SEQ ID NO: 5 - protein, 117 aa, Artificial Sequence
  synthetic construct
EVQLLESGGGLVQPGGSLRLSCAASGFTFSSYYMSWVRQAPGKGLEWVSAISGSGGSTYYADSVKGRFTISRDNSKNTLYLQMNSLRAEDTAVYYCARYARTAFDLWGQGTLVTVSS

SEQ ID NO: 6 - protein, 117 aa, Artificial Sequence
  synthetic construct
EVQLLESGGGLVQPGGSLRLSCAASGFSFSSFYFSWVRQAPGKGLEWVSAISGNGRSTYYADSVKGRFTISRDNSKNTLYLQMNSLRAEDTAVYYCARYYNTGFDLWGQGTLVTVSS

SEQ ID NO: 7 - protein, 117 aa, Artificial Sequence
  synthetic construct
EVQLLESGGGLVQPGGSLRLSCAASGFTFSSYYMSWVRQAPGKGLEWVSAISGNGKSTYYADSVKGRFTISRDNSKNTLYLQMNSLRAEDTAVYYCARYYNTGFDLWGQGTLVTVSS

SEQ ID NO: 8 - protein, 107 aa, Artificial Sequence
  synthetic construct
DIVMTQSPSSLSASVGDRVTITCQASEAIYGYLNWYQQKPGKAPKLLIYAASSLPIGVPSRFSGSGSGTDFTLTISSLQPEDFATYYCQQAYGFPPTFGQGTKLEIK

SEQ ID NO: 9 - protein, 107 aa, Artificial Sequence; identical to SEQ ID NO: 8
  synthetic construct

SEQ ID NO: 10 - protein, 107 aa, Artificial Sequence
  synthetic construct
DIVMTQSPSSLSASVGDGVTITCQASQDIYNYLNWYQQKPGKAPKLLIYYASSIVSGVPSRFSGSGSGTDFTLTISSLQPEDFATYYCQQASSFPPTFGQGTKLEIK

SEQ ID NO: 11 - protein, 453 aa, Artificial Sequence
  synthetic construct
QVQLVQSGAEVKKPGSSVKVSCKASGGTFSSYAISWVRQAPGQGLEWMGGIIPIFGTANYAQKFQGRVTITADKSTSTAYMELSSLRSEDTAVYYCARSPDYSPYYYYGMDVWGQGTTVTVSSASTKGPSVFPLAPSSKSTSGGTAALGCLVKDYFPEPVTVSWNSGALTSGVHTFPAVLQSSGLYSLKSVVTVPSSSLGTQTYICNVNHKPSNTKVDKRVEPKSCDKTHTCPPCPAPEAAGGPSVFLFPPKPKDTLMISRTPEVTCVVVSVSHEDPEVKFNWYVDGVEVHNAKTKPREEQYNSTYRVVSVLTVLHQDWLNGKEYKCKVSNKALPAPIEKTISKAKGQPREPQVYVLPPSRDELTKNQVSLLCLVKGFYPSDIAVEWESNGQPENNYLTWPPVLDSDGSFFLYSKLTVDKSRWQQGNVFSCSVMHEALHNHYTQKSLSLSPGK

SEQ ID NO: 12 - protein, 216 aa, Artificial Sequence
  synthetic construct
QSVLTQPPSASGTPGQRVTISCSGSSSNIGSNTVNWYQQLPGTAPKLLIYGNSNRPSGVPDRFSGSKSGTSASLAISGLQSEDEADYYCQSYDSSLSGSVFGGGIKLTVLGQPKAAPSVTLFPPSSEELQANKATLVCLISDFYPGAVTVAWKADSSPVKAGVETTTPSKQSNNKYAAESELSLTPEQWKSHRSYSCQVTHEGSTVEKTVAPAECS

SEQ ID NO: 13 - protein, 447 aa, Artificial Sequence
  synthetic construct
EVQLLESGGGLVQPGGSLRLSCAASGFTFSSYYMSWVRQAPGKGLEWVSAISGSGGSTYYADSVKGRFTISRDNSKNTLYLQMNSLRAEDTAVYYCARYARTAFDLWGQGTLVTVSSASTKGPSVFPEAPSSKSTSGGTAALGCLVTDYFPEPVTVSWNSGALTSGVHTFPAVLESSGLYSLWSVVTVPSSSLGTQTYICNVNHKPSNTKVDKRVEPKSCDKTHTCPPCPAPEAAGGPSVFLFPPKPKDTLMISRTPEVTCVVVSVSHEDPEVKFNWYVDGVEVHNAKTKPREEQYNSTYRVVSVLTVLHQDWLNGKEYKCKVSNKALPAPIEKTISKAKGQPREPQVYVYPPSRDELTKNQVSLTCLVKGFYPSDIAVEWESNGQPENNYKTTPPVLDSDGSFALVSKLTVDKSRWQQGNVFSCSVMHEALHNHYTQKSLSLSPGK

SEQ ID NO: 14 - protein, 447 aa, Artificial Sequence
  synthetic construct
EVQLLESGGGLVQPGGSLRLSCAASGFSFSSFYFSWVRQAPGKGLEWVSAISGNGRSTYYADSVKGRFTISRDNSKNTLYLQMNSLRAEDTAVYYCARYYNTGFDLWGQGTLVTVSSASTKGPSVFPEAPSSKSTSGGTAALGCLVTDYFPEPVTVSWNSGALTSGVHTFPAVLESSGLYSLWSVVTVPSSSLGTQTYICNVNHKPSNTKVDKRVEPKSCDKTHTCPPCPAPEAAGGPSVFLFPPKPKDTLMISRTPEVTCVVVSVSHEDPEVKFNWYVDGVEVHNAKTKPREEQYNSTYRVVSVLTVLHQDWLNGKEYKCKVSNKALPAPIEKTISKAKGQPREPQVYVYPPSRDELTKNQVSLTCLVKGFYPSDIAVEWESNGQPENNYKTTPPVLDSDGSFALVSKLTVDKSRWQQGNVFSCSVMHEALHNHYTQKSLSLSPGK

SEQ ID NO: 15 - protein, 447 aa, Artificial Sequence
  synthetic construct
EVQLLESGGGLVQPGGSLRLSCAASGFTFSSYYMSWVRQAPGKGLEWVSAISGNGKSTYYADSVKGRFTISRDNSKNTLYLQMNSLRAEDTAVYYCARYYNTGFDLWGQGTLVTVSSASTKGPSVFPEAPSSKSTSGGTAALGCLVTDYFPEPVTVSWNSGALTSGVHTFPAVLESSGLYSLWSVVTVPSSSLGTQTYICNVNHKPSNTKVDKRVEPKSCDKTHTCPPCPAPEAAGGPSVFLFPPKPKDTLMISRTPEVTCVVVSVSHEDPEVKFNWYVDGVEVHNAKTKPREEQYNSTYRVVSVLTVLHQDWLNGKEYKCKVSNKALPAPIEKTISKAKGQPREPQVYVYPPSRDELTKNQVSLTCLVKGFYPSDIAVEWESNGQPENNYKTTPPVLDSDGSFALVSKLTVDKSRWQQGNVFSCSVMHEALHNHYTQKSLSLSPGK

SEQ ID NO: 16 - protein, 214 aa, Artificial Sequence
  synthetic construct
DIVMTQSPSSLSASVGDGVTITCQASQDIYNYLNWYQQKPGKAPKLLIYAASSLQSGVPSRFSGSGSGTDFTLTISSLQPEDFATYYCQQANSFPPTFGQGTKLEIKRTVAAPSVFIFPPSDEQLKSGTARVGCLLNNFYPREAKVQWKVDNALQSGNSQESVTEQDSKDSTYSLRSALTLSKADYEKHKVYACEVTHQGLSSPVTKSFNRGEC

SEQ ID NO: 17 - protein, 214 aa, Artificial Sequence
  synthetic construct
DIVMTQSPSSLSASVGDRVTITCQASEAIYGYLNWYQQKPGKAPKLLIYAASSLPIGVPSRFSGSGSGTDFTLTISSLQPEDFATYYCQQAYGFPPTFGQGTKLEIKRTVAAPSVFIFPPSDEQLKSGTARVGCLLNNFYPREAKVQWKVDNALQSGNSQESVTEQDSKDSTYSLRSALTLSKADYEKHKVYACEVTHQGLSSPVTKSFNRGEC

SEQ ID NO: 18 - protein, 214 aa, Artificial Sequence
  synthetic construct
DIVMTQSPSSLSASVGDGVTITCQASQDIYNYLNWYQQKPGKAPKLLIYYASSIVSGVPSRFSGSGSGTDFTLTISSLQPEDFATYYCQQASSFPPTFGQGTKLEIKRTVAAPSVFIFPPSDEQLKSGTARVGCLLNNFYPREAKVQWKVDNALQSGNSQESVTEQDSKDSTYSLRSALTLSKADYEKHKVYACEVTHQGLSSPVTKSFNRGEC

SEQ ID NO: 19 - protein, 63 aa, Artificial Sequence
  synthetic construct
GPSVFPLAPSSKSTSGGTAALGCLVKDYFPEPVTVSWNSGALTSGVHTFPAVLQSSGLYSLKS

SEQ ID NO: 20 - protein, 35 aa, Artificial Sequence
  synthetic construct
APEAAGGPSVFLFPPKPKDTLMISRTPEVTCVVVS

SEQ ID NO: 21 - protein, 11 aa, Artificial Sequence
  synthetic construct
SNKALPAPIEK

SEQ ID NO: 22 - protein, 61 aa, Artificial Sequence
  synthetic construct
REPQVYVLPPSRDELTKNQVSLLCLVKGFYPSDIAVEWESNGQPENNYLTWPPVLDSDGSF

SEQ ID NO: 23 - protein, 63 aa, Artificial Sequence
  synthetic construct
EAPSSKSTSGGTAALGCLVTDYFPEPVTVSWNSGALTSGVHTFPAVLESSGLYSLWSVVTVPS

SEQ ID NO: 24 - protein, 35 aa, Artificial Sequence; identical to SEQ ID NO: 20
  synthetic construct

SEQ ID NO: 25 - protein, 11 aa, Artificial Sequence
  synthetic construct
APIEKTISKAK

SEQ ID NO: 26 - protein, 61 aa, Artificial Sequence
  synthetic construct
VYPPSRDELTKNQVSLTCLVKGFYPSDIAVEWESNGQPENNYKTTPPVLDSDGSFALVSKL

SEQ ID NO: 27 - protein, 51 aa, Artificial Sequence
  synthetic construct
ANKATLVCLISDFYPGAVTVAWKADSSPVKAGVETTTPSKQSNNKYAAESE

SEQ ID NO: 28 - protein, 51 aa, Artificial Sequence
  synthetic construct
RVGCLLNNFYPREAKVQWKVDNALQSGNSQESVTEQDSKDSTYSLRSALTL

SEQ ID NO: 29 - DNA, 787 bp, Artificial Sequence
  synthetic construct
cagtccgtcctgactcagccaccttccgctagcggtacccccggccagagagtgacaatctcatgctccggttccagctctaacattggctctaacactgtcaattggtaccagcagctgccaggaaccgcaccaaagctgctgatctatggaaactcaaataggcctagcggggtgccagaccggtttagcggatctaaaagtgggacttcagcttccctggcaatttctggactgcagagtgaggacgaagctgattactattgccagtcctacgatagttcactgagcggttccgtgttcggcggagggatcaagctgacagtcctgggccagcccaaggtgagttctagaggatccatctgggataagcatgctgttttctgtctgtccctaacatgccctgtgattatccgcaaacaacacacccaagggcagaactttgttacttaaacaccatcctgtttgcttctttcctcaggccgctccttccgtgactctgtttcccccttccagcgaggaactgcaggccaataaggccaccctggtgtgcctgattagcgacttctatcctggagctgtgacagtcgcatggaaggccgattctagtccagtgaaagcaggggtcgagaccacaactccctccaagcagagcaacaacaagtacgcagccgagtctgaactgagtctgaccccagaacagtggaagtcccacaggagttattcatgccaggtgacccatgagggctccacagtggagaagaccgtggcccctgctgagtgtagc

SEQ ID NO: 30 - DNA, 642 bp, Artificial Sequence
  synthetic construct
gacatcgtgatgacccagtccccttccagcctgtctgcctccgtgggcgacggagtgaccatcacatgccaggctagccaggatatctacaactatctgaattggtaccagcagaagcctggcaaggccccaaagctgctgatctattacgcttcttccatcgtgtctggagtgccatccaggttcagcggatctggatccggaaccgactttaccctgacaatcagctctctgcagcctgaggatttcgccacatactattgccagcaggcttcctctttcccccctacctttggccagggcacaaagctggagatcaagagaaccgtggccgctccatccgtgttcatctttccacccagcgacgagcagctgaagtctggcacagctagggtgggctgtctgctgaacaacttctacccccgggaggccaaggtgcagtggaaggtggataacgctctgcagagcggcaattctcaggagtccgtgaccgagcaggacagcaaggattctacatattccctgagaagcgccctgacactgagcaaggccgattacgagaagcacaaggtgtatgcttgcgaggtgacccatcagggcctgtccagcccagtgacaaagtctttcaatcgcggcgagtgt

SEQ ID NO: 31 - DNA, 1359 bp, Artificial Sequence
  synthetic construct
caggtccagctggtgcagagcggagccgaagtgaagaaacccggtagcagcgtcaaagtgtcatgtaaagcctcagggggaacattctccagctacgccatctcctgggtgagacaggctccaggacagggactggagtggatgggaggaatcatccctatcttcggcaccgccaactacgctcagaagtttcagggccgcgtgaccatcacagccgacaagagcacctctacagcttatatggagctgtcttccctgagaagcgaggatacagccgtgtactattgcgctcgctcccccgactacagcccttactattactatggcatggacgtgtggggccagggcaccacagtgaccgtgagctctgctagcacaaagggcccatccgtgttcccactggctccatccagcaagtccaccagcggaggaacagccgctctgggctgtctggtgaaggactatttcccagagccagtgaccgtgtcctggaacagcggcgccctgacctctggagtgcacacatttcccgctgtgctgcagtcttccggcctgtactctctgaagtccgtggtgaccgtgcctagctcttccctgggcacccagacatatatctgcaacgtgaatcacaagccttccaatacaaaggtggacaagagggtggagccaaagagctgtgataagacccatacatgccccccttgtcctgctccagaggctgctggaggaccaagcgtgttcctgtttccacccaagcccaaggacaccctgatgatctctaggacccctgaggtgacatgcgtggtggtgtccgtgtcccacgaggacccagaggtgaagtttaactggtacgtggatggcgtggaggtgcataatgctaagaccaagcctagggaggagcagtacaacagcacctatcgggtggtgtctgtgctgacagtgctgcatcaggattggctgaacggcaaggagtataagtgcaaggtgtctaataaggccctgcccgctcctatcgagaagaccatctccaaggccaagggccagcctagggagccacaggtgtacgtgctgcctccaagccgggacgagctgacaaagaaccaggtgtctctgctgtgcctggtgaagggcttctatccatctgatatcgctgtggagtgggagtccaatggccagcccgagaacaattacctgacctggccccctgtgctggacagcgatggctctttctttctgtattccaagctgacagtggataagagccggtggcagcagggcaacgtgttctcctgttctgtgatgcacgaggcactgcacaatcattacacccagaaatccctgtcactgagccccggcaag

SEQ ID NO: 32 - DNA, 1341 bp, Artificial Sequence
  synthetic construct
gaggtgcagctgctggagtctggggggggtctggtgcagcccgggggtagcctgcgtctgtcttgtgccgcctctgggtttactttttccagctactatatgagctgggtgagacaggctcctggcaagggcctggagtgggtgtctgccatcagcggcaacggcaaatctacctactatgctgactccgtgaagggcagattcaccatcagccgcgataactctaagaatacactgtacctgcagatgaacagcctgcgcgctgaggacaccgccgtgtactattgcgccagatattataacacaggcttcgatctgtggggccagggcaccctggtgacagtgtcttccgctagcaccaagggcccaagcgtgtttccagaggctccaagctctaagtccaccagcggaggaacagccgctctgggctgtctggtgaccgactacttcccagagcccgtgacagtgtcctggaacagcggcgctctgacctctggcgtgcacacatttccagccgtgctggagtccagcggcctgtactccctgtggtccgtggtgaccgtgcccagctcttccctgggcacccagacatatatctgcaacgtgaatcacaagccatccaatacaaaggtggacaagagggtggagcccaagagctgtgataagacccatacatgccccccttgtcctgctccagaggctgctggaggaccatccgtgttcctgtttccacccaagcctaaggacaccctgatgatcagcaggaccccagaggtgacatgcgtggtggtgtccgtgtcccacgaggaccctgaggtgaagttcaactggtacgtggatggcgtggaggtgcataatgctaagacaaagcccagggaggagcagtacaacagcacctatcgggtggtgtctgtgctgacagtgctgcatcaggattggctgaacggcaaggagtataagtgcaaggtgtctaataaggctctgcccgcccctatcgagaagaccatctccaaggccaagggccagcctagagagccacaggtgtacgtgtatcctccaagccgcgacgagctgaccaagaaccaggtgtctctgacatgtctggtgaagggcttttacccttctgatatcgctgtggagtgggagtccaatggccagccagagaacaattataagaccacaccccctgtgctggactctgatggctccttcgccctggtgtccaagctgaccgtggataagagcaggtggcagcagggcaacgtgttctcctgttctgtgatgcacgaggcactgcacaaccattacacccagaagtccctgtccctgagccccggcaaa